European Patent Specification EP 3 910 075 B1, published December 11, 2024. Title: METHODS AND COMPOSITIONS FOR DETECTING BACTERIAL NUCLEIC ACID AND DIAGNOSING BACTERIAL VAGINOSIS. Applicant: GEN-PROBE INCORPORATED EATON, Barbara L. GETMAN, Damon K. PAWLOWSKI, Traci. Application To Be Assigned. The sequence listing filed with the application follows.

SEQUENCE LISTING (88 sequences)

SEQ ID NO: 1 - DNA, 1518 bp, Lactobacillus crispatus
  ref <308>: GenBank/NR_041800.1 GI:343201103
  ref <309>: 2011-08-10
  ref <313>: (1)..(1518)
gacgaacgctggcggcgtgcctaatacatgcaagtcgagcgagcggaactaacagatttacttcggtaatgacgttaggaaagcgagcggcggatgggtgagtaacacgtggggaacctgccccatagtctgggataccacttggaaacaggtgctaataccggataagaaagcagatcgcatgatcagcttttaaaaggcggcgtaagctgtcgctatgggatggccccgcggtgcattagctagttggtaaggtaaaggcttaccaaggcgatgatgcatagccgagttgagagactgatcggccacattgggactgagacacggcccaaactcctacgggaggcagcagtagggaatcttccacaatggacgcaagtctgatggagcaacgccgcgtgagtgaagaaggttttcggatcgtaaagctctgttgttggtgaagaaggatagaggtagtaactggcctttatttgacggtaatcaaccagaaagtcacggctaactacgtgccagcagccgcggtaatacgtaggtggcaagcgttgtccggatttattgggcgtaaagcgagcgcaggcggaagaataagtctgatgtgaaagccctcggcttaaccgaggaactgcatcggaaactgtttttcttgagtgcagaagaggagagtggaactccatgtgtagcggtggaatgcgtagatatatggaagaacaccagtggcgaaggcggctctctggtctgcaactgacgctgaggctcgaaagcatgggtagcgaacaggattagataccctggtagtccatgccgtaaacgatgagtgctaagtgttgggaggtttccgcctctcagtgctgcagctaacgcattaagcactccgcctggggagtacgaccgcaaggttgaaactcaaaggaattgacgggggcccgcacaagcggtggagcatgtggtttaattcgaagcaacgcgaagaaccttaccaggtcttgacatctagtgccatttgtagagatacaaagttcccttcggggacgctaagacaggtggtgcatggctgtcgtcagctcgtgtcgtgagatgttgggttaagtcccgcaacgagcgcaacccttgttattagttgccagcattaagttgggcactctaatgagactgccggtgacaaaccggaggaaggtggggatgacgtcaagtcatcatgccccttatgacctgggctacacacgtgctacaatgggcagtacaacgagaagcgagcctgcgaaggcaagcgaatctctgaaagctgttctcagttcggactgcagtctgcaactcgactgcacgaagctggaatcgctagtaatcgcggatcagcacgccgcggtgaatacgttcccgggccttgtacacaccgcccgtcacaccatgggagtctgcaatgcccaaagccggtggcctaaccttcgggaaggagccgtctaaggcagggcagatgactggggtgaagtcgtaacaaggtagccgtaggagaactgc

SEQ ID NO: 2 - DNA, 1529 bp, Lactobacillus gasseri
  ref <308>: GenBank/HE573914.1 GI:341599788
  ref <309>: 2011-07-25
  ref <313>: (1)..(1529)
ctgcggcgtgcctaatacatgcaagtcgagcgagcttgcctagatgaatttggtgcttgcaccagatgaaactagatacaagcgagcggcggacgggtgagtaacacgtgggtaacctgcccaagagactgggataacacctggaaacagatgctaataccggataacaacactagacgcatgtctagagtttaaaagatggttctgctatcactcttggatggacctgcggtgcattagctagttggtaaggtaacggcttaccaaggcaatgatgcatagccgagttgagagactgatcggccacattgggactgagacacggcccaaactcctacgggaggcagcagtagggaatcttccacaatggacgcaagtctgatggagcaacgccgcgtgagtgaagaagggtttcggctcgtaaagctctgttggtagtgaagaaagatagaggtagtaactggcctttatttgacggtaattacttagaaagtcacggctaactacgtgccagcagccgcggtaatacgtaggtggcaagcgttgtccggatttattgggcgtaaagcgagtgcaggcggttcaataagtctgatgtgaaagccttcggctcaaccggagaattgcatcagaaactgttgaacttgagtgcagaagaggagagtggaactccatgtgtagcggtggaatgcgtagatatatggaagaacaccagtggcgaaggcggctctctggtctgcaactgacgctgaggctcgaaagcatgggtagcgaacaggattagataccctggtagtccatgccgtaaacgatgagtgctaagtgttgggaggtttccgcctctcagtgctgcagctaacgcattaagcactccgcctggggagtacgaccgcaaggttgaaactcaaaggaattgacgggggcccgcacaagcggtggagcatgtggtttaattcgaagcaacgcgaagaaccttaccaggtcttgacatccagtgcaaacctaagagattaggtgttcccttcggggacgctgagacaggtggtgcatggctgtcgtcagctcgtgtcgtgagatgttgggttaagtcccgcaacgagcgcaacccttgtcattagttgccatcattaagttgggcactctaatgagactgccggtgacaaaccggaggaaggtggggatgacgtcaagtcatcatgccccttatgacctgggctacacacgtgctacaatggacggtacaacgagaagcgaacctgcgaaggcaagcggatctctgaaagccgttctcagttcggactgtaggctgcaactcgcctacacgaagctggaatcgctagtaatcgcggatcagcacgccgcggtgaatacgttcccgggccttgtacacaccgcccgtcacaccatgagagtctgtaacacccaaagccggtgggataacctttataggagtcagccgtctaaggtaggacagatgattagggtgaagtcgtaacaaggtagccgtaggagaacctgcggttggatca

SEQ ID NO: 3 - DNA, 1475 bp, Gardnerella vaginalis
  misc_feature (60)..(60): n is a, c, g, or t
  misc_feature (340)..(340): n is a, c, g, or t
  misc_feature (399)..(399): n is a, c, g, or t
  misc_feature (612)..(612): n is a, c, g, or t
  misc_feature (916)..(916): n is a, c, g, or t
  misc_feature (951)..(951): n is a, c, g, or t
  misc_feature (1012)..(1012): n is a, c, g, or t
  misc_feature (1156)..(1156): n is a, c, g, or t
  misc_feature (1171)..(1171): n is a, c, g, or t
  misc_feature (1277)..(1277): n is a, c, g, or t
  ref <308>: GenBank/NR_044694.2 GI:545589071
  ref <309>: 2013-09-24
  ref <313>: (1)..(1475)
tttcgtggagggttcgattctggctcaggatgaacgctggcggcgtgcttaacacatgcnagtcgaacgggatctgaccagcttgctggttggtgagagtggcgaacgggtgagtaatgcgtgaccaacctgccccatgctccagaatagctcttggaaacgggtggtaatgctggatgctccaacttgacgcatgtcttgttgggaaagtgtttagtggcatgggatggggtcgcgtcctatcagcttgtaggcggggtaatggcccacctaggcttcgacgggtagccggcctgagagggcggacggccacattgggactgagatacggcccagactnctacgggaggcagcagtggggaatattgcgcaatgggggaaaccctgacgcagcgacgncgcgtgcgggatgaaggccttcgggttgtaaaccgcttttgattgggagcaagccttttgggtgagtgtacctttcgaataagcgccggctaactacgtgccagcagccgcggtaatacgtagggcgcaagcgttatccggaattattgggcgtaaagagcttgtaggcggttcgtcgcgtctggtgtgaaagcccatcgcttaacggtgggnttgcgccgggtacgggcgggctagagtgcagtaggggagactggaattctcggtgtaacggtggaatgtgtagatatcgggaagaacaccaatggcgaaggcaggtctctgggctgttactgacgctgagaagcgaaagcgtggggagcgaacaggattagataccctggtagtccacgccgtaaacggtggacgctggatgtggggcccattccacgggttctgtgtcggagctaacgcgttaagcgtcccgcctggggagtacggccgcaaggctaaaactcaaagaaattgacgggggccngcacaagcggcggagcatgcggattaattcgatgnaacgcgaagaaccttacctgggcttgacatgtgcctgacgactgcagagatgtggtttccnttcggggcaggttcacaggtggtgcatggtcgtcgtcagctcgtgtcgtgagatgttgggttaagtcccgcaacgagcgcaaccctcgccctgtgttgccagcgggttatgccgggaactcacgggggaccgccggggttaccncggaggaaggtgggnatgacgtcagatcatcatgccccttacgtccagggcttcacgcatgctacaatggccagtacaacgggttgcttcatggtgacatggtgctaatcccttaaaactngtctcagttcggatcgtagtctgcaactcgactacgtgaaggcggagtcgctagtaatcgcgaatcagcaacgtcgcggtgaatgcgttcccgggccttgtacacaccgcccgtcaagtcatgaaagtgggcagcacccgaagccggtggcctaacccttttgggatggagccgtctaaggtgaggctcgtgattggg

SEQ ID NO: 4 - DNA, 1000 bp, Uncultured Eggerthella sp. clone 123-f2 68
  ref <308>: GenBank/AY738656.1  GI:52222145
  ref <309>: 2005-11-02
  ref <313>: (1)..(1000)
tggggaatattgcgcaatgggggaaaccctgacgcagcaacgccgcgtgcgggatgaaggccttcgggttgtaaaccgctttcagcagggaagacatcgacggtacctgcagaagaagccccggctaactacgtgccagcagccgcggtaatacgtagggggcgagcgttatccggattcattgggcgtaaagcgcgcgcaggcggttgctcaagcggaacctctaatctcggggcttaacctcgagccgggttccgaactggacgactcgagtgcggtagaggcagatggaattcccggtgtagcggtggaatgcgcagatatcgggaagaacaccaacggcgaaggcagtctgctgggccgtcactgacgctgaggcgcgaaagctgggggagcgaacaggattagataccctggtagtcccagccgtaaacgatgagcgctgggtgtgggagattacatcttccgtgccgaagctaacgcattaagcgctccgcctggggagtacggccgcaaggctaaaactcaaaggaattgacgggggcccgcacaagcagcggagcatgtggcttaattcgaagcaacgcgaagaaccttaccagggcttgacatgtaggtgaagcggcggaaacgtcgtggccgaaaggagcctacacaggtggtgcatggctgtcgtcagctcgtgtcgtgagatgttgggttaagtcccgcaacgagcgcaacccctgccccgtgttaccagcatttagttggggactcgcgggggactgccggcgtcaagccggaggaaggcggggatgacgtcaagtcatcatgccccttatgccctgggccgcacacgtgctacaatggccggcacagcgggctgcaacctagcgataggaagcgaatcccgtaaagccggtcccagttcggattggaggctgaaacccgcctccatgaagccggagttgctagtaatcgcggatcagcacgccgcggtgaatgcgttcccgggcct

SEQ ID NO: 5 - DNA, 45 bp, Artificial Sequence
  Synthetic Oligomer
  misc_feature (13)..(45): Immobilized probe-binding region: Tail
ucuguuaguucctttaaaaaaaaaaaaaaaaaaaaaaaaaaaaaa

SEQ ID NO: 6 - DNA, 16 bp, Artificial Sequence
  Synthetic Oligomer
cggatgggtgagtaac

SEQ ID NO: 7 - DNA, 45 bp, Artificial Sequence
  Synthetic Oligomer
  promoter (1)..(27)
aatttaatacgactcactatagggagataagcccttaccttacca

SEQ ID NO: 8 - DNA, 45 bp, Artificial Sequence
  Synthetic Oligomer
  promoter (1)..(27)
aatttaatacgactcactatagggagataagccgttaccttacca

SEQ ID NO: 9 - DNA, 26 bp, Artificial Sequence
  Synthetic Oligomer
gucugggauaccacuuggaaacagac

SEQ ID NO: 10 - DNA, 21 bp, Artificial Sequence
  Synthetic Oligomer
cacucacgcaugucuagagug

SEQ ID NO: 11 - DNA, 50 bp, Artificial Sequence
  Synthetic Oligomer
  misc_feature (18)..(50): Immobilized probe-binding region: Tail
caugcuccgccgcuugutttaaaaaaaaaaaaaaaaaaaaaaaaaaaaaa

SEQ ID NO: 12 - DNA, 25 bp, Artificial Sequence
  Synthetic Oligomer
cttacctgggcttgacatgtgcctg

SEQ ID NO: 13 - DNA, 45 bp, Artificial Sequence
  Synthetic Oligomer
  promoter (1)..(27)
aatttaatacgactcactatagggagacaccacctgtgaacctgc

SEQ ID NO: 14 - DNA, 24 bp, Artificial Sequence
  Synthetic Oligomer
ccugcagagaugugguuucgcagg

SEQ ID NO: 15 - DNA, 54 bp, Artificial Sequence
  Synthetic Oligomer
  misc_feature (22)..(54): Immobilized probe-binding region: Tail
guaccgucgaugucuucccugtttaaaaaaaaaaaaaaaaaaaaaaaaaaaaaa

SEQ ID NO: 16 - DNA, 16 bp, Artificial Sequence
  Synthetic Oligomer
agcgttatccggattc

SEQ ID NO: 17 - DNA, 51 bp, Artificial Sequence
  Synthetic Oligomer
  promoter (1)..(27)
aatttaatacgactcactatagggagattcggaacccggctcgaggttaag

SEQ ID NO: 18 - DNA, 24 bp, Artificial Sequence
  Synthetic Oligomer
ccgcucaggcgguugcucaagcgg

SEQ ID NO: 19 - DNA, 20 bp, Artificial Sequence
  Synthetic Oligomer
ggattcattgggcgtaaagc

SEQ ID NO: 20 - DNA, 17 bp, Artificial Sequence
  Synthetic Oligomer
gcgttatccggattcat

SEQ ID NO: 21 - DNA, 45 bp, Artificial Sequence
  Synthetic Oligomer
  promoter (1)..(27)
aatttaatacgactcactatagggagataagcctttaccttacca

SEQ ID NO: 22 - DNA, 46 bp, Artificial Sequence
  Synthetic Oligomer
  promoter (1)..(27)
aatttaatacgactcactatagggagaatacgacagcttacgccgc

SEQ ID NO: 23 - DNA, 51 bp, Artificial Sequence
  Synthetic Oligomer
  promoter (1)..(27)
aatttaatacgactcactatagggagatatctgcgcatttcaccgctacac

SEQ ID NO: 24 - DNA, 45 bp, Artificial Sequence
  Synthetic Oligomer
  promoter (1)..(27)
aatttaatacgactcactatagggagacgaccatgcaccacctgt

SEQ ID NO: 25 - DNA, 57 bp, Artificial Sequence
  Synthetic Oligomer
  misc_feature (25)..(57): Immobilized probe-binding region: Tail
ggacuaccaggguaucuaauccugtttaaaaaaaaaaaaaaaaaaaaaaaaaaaaaa

SEQ ID NO: 26 - DNA, 52 bp, Artificial Sequence
  Synthetic Oligomer
  misc_feature (20)..(52): Immobilized probe-binding region: Tail
guaggaguuugggccgugutttaaaaaaaaaaaaaaaaaaaaaaaaaaaaaa

SEQ ID NO: 27 - DNA, 53 bp, Artificial Sequence
  Synthetic Oligomer
  misc_feature (21)..(53): Immobilized probe-binding region: Tail
cuuugaguuuuagccuugcgtttaaaaaaaaaaaaaaaaaaaaaaaaaaaaaa

SEQ ID NO: 28 - DNA, 54 bp, Artificial Sequence
  Synthetic Oligomer
  misc_feature (22)..(54): Immobilized probe-binding region: Tail
gcaucgaauuaauccgcaugctttaaaaaaaaaaaaaaaaaaaaaaaaaaaaaa

SEQ ID NO: 29 - DNA, 54 bp, Artificial Sequence
  Synthetic Oligomer
  misc_feature (22)..(54): Immobilized probe-binding region: Tail
guaguuagccggggcuucuuctttaaaaaaaaaaaaaaaaaaaaaaaaaaaaaa

SEQ ID NO: 30 - DNA, 51 bp, Artificial Sequence
  Synthetic Oligomer
  misc_feature (19)..(51): Immobilized probe-binding region: Tail
uacguauuaccgcggcugtttaaaaaaaaaaaaaaaaaaaaaaaaaaaaaa

SEQ ID NO: 31 - DNA, 53 bp, Artificial Sequence
  Synthetic Oligomer
  misc_feature (21)..(53): Immobilized probe-binding region: Tail
cgugucucagucccaaugugtttaaaaaaaaaaaaaaaaaaaaaaaaaaaaaa

SEQ ID NO: 32 - DNA, 51 bp, Artificial Sequence
  Synthetic Oligomer
  misc_feature (19)..(51): Immobilized probe-binding region: Tail
caauguggccgaucaguctttaaaaaaaaaaaaaaaaaaaaaaaaaaaaaa

SEQ ID NO: 33 - DNA, 54 bp, Artificial Sequence
  Synthetic Oligomer
  misc_feature (22)..(54): Immobilized probe-binding region: Tail
ccauuguggaagauucccuactttaaaaaaaaaaaaaaaaaaaaaaaaaaaaaa

SEQ ID NO: 34 - DNA, 52 bp, Artificial Sequence
  Synthetic Oligomer
  misc_feature (20)..(52): Immobilized probe-binding region: Tail
cucgcucgacuugcauguatttaaaaaaaaaaaaaaaaaaaaaaaaaaaaaa

SEQ ID NO: 35 - DNA, 52 bp, Artificial Sequence
  Synthetic Oligomer
  misc_feature (20)..(52): Immobilized probe-binding region: Tail
cuugcauguauuaggcacgtttaaaaaaaaaaaaaaaaaaaaaaaaaaaaaa

SEQ ID NO: 36 - DNA, 53 bp, Artificial Sequence
  Synthetic Oligomer
  misc_feature (21)..(53): Immobilized probe-binding region: Tail
cuuguaucuauguccauucctttaaaaaaaaaaaaaaaaaaaaaaaaaaaaaa

SEQ ID NO: 37 - DNA, 52 bp, Artificial Sequence
  Synthetic Oligomer
  misc_feature (20)..(52): Immobilized probe-binding region: Tail
uggugcaagcaccaaauuctttaaaaaaaaaaaaaaaaaaaaaaaaaaaaaa

SEQ ID NO: 38 - DNA, 49 bp, Artificial Sequence
  Synthetic Oligomer
  misc_feature (17)..(49): Immobilized probe-binding region: Tail
aauucaucuaggcaagtttaaaaaaaaaaaaaaaaaaaaaaaaaaaaaa

SEQ ID NO: 39 - DNA, 49 bp, Artificial Sequence
  Synthetic Oligomer
  misc_feature (17)..(49): Immobilized probe-binding region: Tail
uccuaacgucauuacctttaaaaaaaaaaaaaaaaaaaaaaaaaaaaaa

SEQ ID NO: 40 - DNA, 47 bp, Artificial Sequence
  Synthetic Oligomer
  misc_feature (15)..(47): Immobilized probe-binding region: Tail
uccauuccgaagaatttaaaaaaaaaaaaaaaaaaaaaaaaaaaaaa

SEQ ID NO: 41 - DNA, 52 bp, Artificial Sequence
  Synthetic Oligomer
  misc_feature (20)..(52): Immobilized probe-binding region: Tail
uugcugcgucaggguuucctttaaaaaaaaaaaaaaaaaaaaaaaaaaaaaa

SEQ ID NO: 42 - DNA, 53 bp, Artificial Sequence
  Synthetic Oligomer
  misc_feature (21)..(53): Immobilized probe-binding region: Tail
gaaagcgguuuacaacccgatttaaaaaaaaaaaaaaaaaaaaaaaaaaaaaa

SEQ ID NO: 43 - DNA, 50 bp, Artificial Sequence
  Synthetic Oligomer
  misc_feature (18)..(50): Immobilized probe-binding region: Tail
aaggccuucaucccgcatttaaaaaaaaaaaaaaaaaaaaaaaaaaaaaa

SEQ ID NO: 44 - DNA, 51 bp, Artificial Sequence
  Synthetic Oligomer
  misc_feature (19)..(51): Immobilized probe-binding region: Tail
ucgccguugguguucuuctttaaaaaaaaaaaaaaaaaaaaaaaaaaaaaa

SEQ ID NO: 45 - DNA, 50 bp, Artificial Sequence
  Synthetic Oligomer
  misc_feature (18)..(50): Immobilized probe-binding region: Tail
ugacggcccagcagacutttaaaaaaaaaaaaaaaaaaaaaaaaaaaaaa

SEQ ID NO: 46 - DNA, 53 bp, Artificial Sequence
  Synthetic Oligomer
  misc_feature (21)..(53): Immobilized probe-binding region: Tail
uccuguucgcucccccagcutttaaaaaaaaaaaaaaaaaaaaaaaaaaaaaa

SEQ ID NO: 47 - DNA, 49 bp, Artificial Sequence
  Synthetic Oligomer
  misc_feature (17)..(49): Immobilized probe-binding region: Tail
tcctaacgtcattacctttaaaaaaaaaaaaaaaaaaaaaaaaaaaaaa

SEQ ID NO: 48 - DNA, 54 bp, Artificial Sequence
  Synthetic Oligomer
  misc_feature (22)..(54): Immobilized probe-binding region: Tail
gtaccgtcgatgtcttccctgtttaaaaaaaaaaaaaaaaaaaaaaaaaaaaaa

SEQ ID NO: 49 - DNA, 47 bp, Artificial Sequence
  Synthetic Oligomer
  misc_feature (15)..(47): Immobilized probe-binding region: Tail
cagcgcucaucguutttaaaaaaaaaaaaaaaaaaaaaaaaaaaaaa

SEQ ID NO: 50 - DNA, 50 bp, Artificial Sequence
  Synthetic Oligomer
  misc_feature (18)..(50): Immobilized probe-binding region: Tail
acggaagauguaaucuctttaaaaaaaaaaaaaaaaaaaaaaaaaaaaaa

SEQ ID NO: 51 - DNA, 48 bp, Artificial Sequence
  Synthetic Oligomer
  misc_feature (16)..(48): Immobilized probe-binding region: Tail
gauguaaucucccactttaaaaaaaaaaaaaaaaaaaaaaaaaaaaaa

SEQ ID NO: 52 - DNA, 45 bp, Artificial Sequence
  Synthetic Oligomer
  misc_feature (13)..(45): Immobilized probe-binding region: Tail
ccauuccgaagatttaaaaaaaaaaaaaaaaaaaaaaaaaaaaaa

SEQ ID NO: 53 - DNA, 44 bp, Artificial Sequence
  Synthetic Oligomer
  misc_feature (12)..(44): Immobilized probe-binding region: Tail
aguuucaucugtttaaaaaaaaaaaaaaaaaaaaaaaaaaaaaa

SEQ ID NO: 54 - DNA, 45 bp, Artificial Sequence
  Synthetic Oligomer
  misc_feature (13)..(45): Immobilized probe-binding region: Tail
ccgaagaauuuctttaaaaaaaaaaaaaaaaaaaaaaaaaaaaaa

SEQ ID NO: 55 - DNA, 43 bp, Artificial Sequence
  Synthetic Oligomer
  misc_feature (11)..(43): Immobilized probe-binding region: Tail
uucaauaggctttaaaaaaaaaaaaaaaaaaaaaaaaaaaaaa

SEQ ID NO: 56 - DNA, 43 bp, Artificial Sequence
  Synthetic Oligomer
  misc_feature (11)..(43): Immobilized probe-binding region: Tail
cgucauuacctttaaaaaaaaaaaaaaaaaaaaaaaaaaaaaa

SEQ ID NO: 57 - DNA, 45 bp, Artificial Sequence
  Synthetic Oligomer
  misc_feature (13)..(45): Immobilized probe-binding region: Tail
ccaaauucaucutttaaaaaaaaaaaaaaaaaaaaaaaaaaaaaa

SEQ ID NO: 58 - DNA, 45 bp, Artificial Sequence
  Synthetic Oligomer
  misc_feature (13)..(45): Immobilized probe-binding region: Tail
aacgucauuacctttaaaaaaaaaaaaaaaaaaaaaaaaaaaaaa

SEQ ID NO: 59 - DNA, 45 bp, Artificial Sequence
  Synthetic Oligomer
  misc_feature (13)..(45): Immobilized probe-binding region: Tail
uuuccuaacguctttaaaaaaaaaaaaaaaaaaaaaaaaaaaaaa

SEQ ID NO: 60 - DNA, 24 bp, Artificial Sequence
  Synthetic Oligomer
ccugcagagaugugguuucgcagg

SEQ ID NO: 61 - DNA, 26 bp, Artificial Sequence
  Synthetic Oligomer
cugggauaccacuuggaaacacccag

SEQ ID NO: 62 - DNA, 20 bp, Artificial Sequence
  Synthetic Oligomer
ucugggauaccacuuccaga

SEQ ID NO: 63 - DNA, 24 bp, Artificial Sequence
  Synthetic Oligomer
ccugcagagaugugguuucgcagg

SEQ ID NO: 64 - DNA, 24 bp, Artificial Sequence
  Synthetic Oligomer
gguucugcuaucacucuuggaacc

SEQ ID NO: 65 - DNA, 20 bp, Artificial Sequence
  Synthetic Oligomer
acgcaugucuagaguugcgu

SEQ ID NO: 66 - DNA, 21 bp, Artificial Sequence
  Synthetic Oligomer
agacgcaugucuagagcgucu

SEQ ID NO: 67 - DNA, 27 bp, Artificial Sequence
  Synthetic Oligomer
gaugcuaauaccggauaacaacgcauc

SEQ ID NO: 68 - DNA, 28 bp, Artificial Sequence
  Synthetic Oligomer
uaccggauaacaacacuagacgccggua

SEQ ID NO: 69 - DNA, 26 bp, Artificial Sequence
  Synthetic Oligomer
gucugggauaccauuuggaaacagac

SEQ ID NO: 70 - DNA, 26 bp, Artificial Sequence
  Synthetic Oligomer
gucugggauaccacuuggaaacagac

SEQ ID NO: 71 - DNA, 26 bp, Artificial Sequence
  Synthetic Oligomer
gucugggauaccacuuggaaacagac

SEQ ID NO: 72 - DNA, 24 bp, Artificial Sequence
  Synthetic Oligomer
gguucugcuaucacucuuggaacc

SEQ ID NO: 73 - DNA, 24 bp, Artificial Sequence
  Synthetic Oligomer
gguucugcuaucacucuuggaacc

SEQ ID NO: 74 - DNA, 18 bp, Artificial Sequence
  Synthetic Oligomer
cgcaugucuagaguugcg

SEQ ID NO: 75 - DNA, 19 bp, Artificial Sequence
  Synthetic Oligomer
acucacgcaugucuagagu

SEQ ID NO: 76 - DNA, 24 bp, Artificial Sequence
  Synthetic Oligomer
gagacgcaugucuagaguugucuc

SEQ ID NO: 77 - DNA, 24 bp, Artificial Sequence
  Synthetic Oligomer
guugcucaagcggaaccucgcaac

SEQ ID NO: 78 - DNA, 24 bp, Artificial Sequence
  Synthetic Oligomer
uugcucaagcggaaccucuagcaa

SEQ ID NO: 79 - DNA, 21 bp, Artificial Sequence
  Synthetic Oligomer
gcucaagcggaaccucugagc

SEQ ID NO: 80 - DNA, 24 bp, Artificial Sequence
  Synthetic Oligomer
agcggaaccucuaaucucgucgcu

SEQ ID NO: 81 - DNA, 24 bp, Artificial Sequence
  Synthetic Oligomer
ccgcucaggcgguugcucaagcgg

SEQ ID NO: 82 - DNA, 24 bp, Artificial Sequence
  Synthetic Oligomer
ccgcucaggcgguugcucaagcgg

SEQ ID NO: 83 - DNA, 24 bp, Artificial Sequence
  Synthetic Oligomer
ccgcucaggcgguugcucaagcgg

SEQ ID NO: 84 - DNA, 24 bp, Artificial Sequence
  Synthetic Oligomer
ccgcucaggcgguugcucaagcgg

SEQ ID NO: 85 - DNA, 24 bp, Artificial Sequence
  Synthetic Oligomer
ccgcucaggcgguugcucaagcgg

SEQ ID NO: 86 - DNA, 24 bp, Artificial Sequence
  Synthetic Oligomer
ccgcucaggcgguugcucaagcgg

SEQ ID NO: 87 - DNA, 24 bp, Artificial Sequence
  Synthetic Oligomer
ccgcucaggcgguugcucaagcgg

SEQ ID NO: 88 - DNA, 1496 bp, Lactobacillus jensenii
  ref <308>: GenBank/NR_025087.1  GI:219857499
  ref <309>: 2009-01-09
  ref <313>: (1)..(1496)
tgcctaatacatgcaagtcgagcgagcttgcctatagaagttcttcggaatggaaatagatacaagctagcggcggatgggtgagtaacgcgtgggtaacctgcccttaagtctgggataccatttggaaacagatgctaataccggataaaagctactttcgcatgaaagaagtttaaaaggcggcgtaagctgtcgtaaaggatggacttgcgatgcattagctagttggtaaggtaacggcttaccaaggctgatgatgcatagccgagttgagagactgatcggccacattgggactgagacacggcccaaactcctacgggaggcagcagtagggaatcttccacaatggacgaaagtctgatggagcaacgccgcgtgagtgaagaaggttttcggatcgtaaagctctgttgttggtgaagaaggatagaggtagtaactggcctttatttgacggtaatcaaccagaaagtcacggctaactacgtgccagcagccgcggtaatacgtaggtggcaagcgttgtccggatttattgggcgtaaagcgagcgcaggcggattgataagtctgatgtgaaagccttcggctcaaccgaagaactgcatcagaaactgtcaatcttgagtgcagaagaggagagtggaactccatgtgtagcggtggaatgcgtagatatatggaagaacaccagtggcgaaggcggctctctggtctgtaactgacgctgaggctcgaaagcatgggtagcgaacaggattagataccctggtagtccatgccgtaaacgatgagtgctaagtgttgggaggtttccgcctctcagtgctgcagctaacgcattaagcactccgcctggggagtacgaccgcaaggttgaaactcaaaggaattgacgggggcccgcacaagcggtggagcatgtggtttaattcgaagcaacgcgaagaaccttaccaggtcttgacatcctttgaccacctaagagattaggttttcccttcggggacaaagagacaggtggtgcatggctgtcgtcagctcgtgtcgtgagatgttgggttaagtcccgcaacgagcgcaacccttgttaatagttgccagcattaagttgggcactctattgagactgccggtgacaaaccggaggaaggtggggatgacgtcaagtcatcatgccccttatgacctgggctacacacgtgctacaatgggcagtacaacgagaagcgaacctgtgaaggcaagcggatctcttaaagctgttctcagttcggactgtaggctgcaactcgcctacacgaagctggaatcgctagtaatcgcggatcagcacgccgcggtgaatacgttcccgggccttgtacacaccgcccgtcacaccatgagagtttgtaacacccaaagtcggtgaggtaacctttggagccagccgcctaaggtgggacagatgattagggtgaagtcgtaacaaggtagccgtaggagaa